European Patent Specification EP 3 998 338 B1, published April 24, 2024. Title: Method of nucleic acid amplification from solid support. Applicant: Tokyo University of Science Foundation. The sequence listing filed with the application follows.

SEQUENCE LISTING (32 sequences)

SEQ ID NO: 1 - DNA, 99 bp, Artificial Sequence
  LibA-BC-linker-UMI-dT27VN
  misc_feature (28)..(39): barcode for bead identification
  misc_feature (63)..(70): unique molecular identifier
  misc_feature (99)..(99): n is A, T, C or G
ctatgcgccttgccagcccgctcagacnnnnnnnnnnnngatggcgcgagggaggcgatacgnnnnnnnntttttttttttttttttttttttttttvn

SEQ ID NO: 2 - DNA, 30 bp, Artificial Sequence
  primer Biosg-LibB-TSO
ctatgcgccttgccagcccgctcagacggg

SEQ ID NO: 3 - DNA, 52 bp, Artificial Sequence
  primer LibB-dT25VN-primer
  misc_feature (52)..(52): n is A, T, C or G
cgtatcgcctccctcgcgccaagtctgtttttttttttttttttttttttvn

SEQ ID NO: 4 - DNA, 27 bp, Artificial Sequence
  primer Biosg-LibA-primer
ctatgcgccttgccagcccgctcagac

SEQ ID NO: 5 - DNA, 27 bp, Artificial Sequence
  primer Biosg-LibB-primer
cgtatcgcctccctcgcgccatcagac

SEQ ID NO: 6 - DNA, 50 bp, Artificial Sequence
  BioEcoP-dT25-adapter
aagcagtggtatcaacgcagagtacttttttttttttttttttttttttt

SEQ ID NO: 7 - DNA, 45 bp, Artificial Sequence
  primer 5'WTA-dT25
gcggctgaagacggcctatgttttttttttttttttttttttttt

SEQ ID NO: 8 - DNA, 30 bp, Artificial Sequence
  primer 5'WTA-dG9
gcggctgaagacggcctatgtggggggggg

SEQ ID NO: 9 - DNA, 21 bp, Artificial Sequence
  primer 5'WTA
gcggctgaagacggcctatgt

SEQ ID NO: 10 - DNA, 23 bp, Artificial Sequence
  primer 3'WTA
aagcagtggtatcaacgcagagt

SEQ ID NO: 11 - DNA, 98 bp, Artificial Sequence
  Rhapsody universal adapter
  misc_feature (21)..(29): CLS1
  misc_feature (42)..(50): CLS2
  misc_feature (64)..(72): CLS3
  misc_feature (73)..(80): n is A, T, C or G
acacgacgctcttccgatctnnnnnnnnnactggcctgcgannnnnnnnnggtagcggtgacannnnnnnnnnnnnnnnntttttttttttttttttt

SEQ ID NO: 12 - DNA, 37 bp, Artificial Sequence
  primer LibA-dG9
ctatgcgccttgccagcccgctcagactggggggggg

SEQ ID NO: 13 - DNA, 28 bp, Artificial Sequence
  primer NH2-LibA
ctatgcgccttgccagcccgctcagact

SEQ ID NO: 14 - DNA, 33 bp, Artificial Sequence
  primer NH2-Universal
acactctttccctacacgacgctcttccgatct

SEQ ID NO: 15 - DNA, 33 bp, Artificial Sequence
  Illumina adapter
gatcggaagagcacacgtctgaactccagtcac

SEQ ID NO: 16 - DNA, 13 bp, Artificial Sequence
  Illumina adapter
gctcttccgatct

SEQ ID NO: 17 - DNA, 57 bp, Artificial Sequence
  primer ILMN_I5_S531
aatgatacggcgaccaccgagatctacaccggcattaacactctttccctacacgac

SEQ ID NO: 18 - DNA, 57 bp, Artificial Sequence
  primer ILMN_I5_S589
aatgatacggcgaccaccgagatctacaccacgcaatacactctttccctacacgac

SEQ ID NO: 19 - DNA, 57 bp, Artificial Sequence
  primer ILMN_I5_S587
aatgatacggcgaccaccgagatctacacggaatgtcacactctttccctacacgac

SEQ ID NO: 20 - DNA, 57 bp, Artificial Sequence
  primer ILMN_I5_S503
aatgatacggcgaccaccgagatctacactggtgaagacactctttccctacacgac

SEQ ID NO: 21 - DNA, 53 bp, Artificial Sequence
  primer ILMN_I7_S771
caagcagaagacggcatacgagattgactgacgtgactggagttcagacgtgt

SEQ ID NO: 22 - DNA, 53 bp, Artificial Sequence
  primer ILMN_I7_S779
caagcagaagacggcatacgagatatggaagggtgactggagttcagacgtgt

SEQ ID NO: 23 - DNA, 53 bp, Artificial Sequence
  primer ILMN_I7_S788
caagcagaagacggcatacgagatgtgttcctgtgactggagttcagacgtgt

SEQ ID NO: 24 - DNA, 53 bp, Artificial Sequence
  primer ILMN_I7_S739
caagcagaagacggcatacgagatgctgtaaggtgactggagttcagacgtgt

SEQ ID NO: 25 - DNA, 82 bp, Artificial Sequence
  Biolegend Hashtag Totalseq-A
  misc_feature (35)..(49): barcode for antibody identification
gtgactggagttcagacgtgtgctcttccgatctnnnnnnnnnnnnnnnbaaaaaaaaaaaaaaaaaaaaaaaaaaaaaaaa

SEQ ID NO: 26 - DNA, 30 bp, Artificial Sequence
  5'BDWTA-dG9
aagcagtggtatcaacgcagaggggggggg

SEQ ID NO: 27 - DNA, 21 bp, Artificial Sequence
  NH2-5'BDWTA
aagcagtggtatcaacgcaga

SEQ ID NO: 28 - DNA, 21 bp, Artificial Sequence
  Hashtag Common
gtgactggagttcagacgtgt

SEQ ID NO: 29 - DNA, 56 bp, Artificial Sequence
  ILMN_UDI0030-I5
aatgatacggcgaccaccgagatctacactgacaagccactctttccctacacgac

SEQ ID NO: 30 - DNA, 57 bp, Artificial Sequence
  ILMN_UDI0033-I5
aatgatacggcgaccaccgagatctacaccctgaactacactctttccctacacgac

SEQ ID NO: 31 - DNA, 53 bp, Artificial Sequence
  ILMN_UDI0030-I7
caagcagaagacggcatacgagattcctgtaagtgactggagttcagacgtgt

SEQ ID NO: 32 - DNA, 53 bp, Artificial Sequence
  ILMN_UDI0033-I7
caagcagaagacggcatacgagatcctcggtagtgactggagttcagacgtgt